European Patent Application EP 4 410 821 A1, published August 7, 2024. Title: Blood Brain Barrier Penetrating Peptide and Use Thereof. Applicant: Seoul National University R&DB Foundation. The sequence listing filed with the application follows.

SEQUENCE LISTING (89 sequences)

SEQ ID NO: 1 - protein, 5 aa, synthetic construct
VPALR

SEQ ID NO: 2 - protein, 16 aa, synthetic construct
LRRERQSRLRRERQSR

SEQ ID NO: 3 - protein, 19 aa, synthetic construct
VPALRRERQSRLRRERQSR

SEQ ID NO: 4 - protein, 7 aa, synthetic construct
HAIYPRH

SEQ ID NO: 5 - protein, 12 aa, synthetic construct
YHFNGCEDPLCR

SEQ ID NO: 6 - protein, 12 aa, synthetic construct
HPWCCGLRLDLR

SEQ ID NO: 7 - protein, 11 aa, synthetic construct
HRRCNKNNKKR

SEQ ID NO: 8 - protein, 11 aa, synthetic construct
HRRCNPNNKKR

SEQ ID NO: 9 - protein, 14 aa, synthetic construct
VSRRRRRRGGRRRR

SEQ ID NO: 10 - protein, 15 aa, synthetic construct
GKCSTRGRKCCRRKK

SEQ ID NO: 11 - protein, 16 aa, synthetic construct
VPALRHRRCNKNNKKR

SEQ ID NO: 12 - protein, 16 aa, synthetic construct
VPALRHRRCNPNNKKR

SEQ ID NO: 13 - protein, 19 aa, synthetic construct
VPALRVSRRRRRRGGRRRR

SEQ ID NO: 14 - protein, 20 aa, synthetic construct
VPALRGKCSTRGRKCCRRKK

SEQ ID NO: 15 - protein, 16 aa, synthetic construct
HRRCNKNNKKRVPALR

SEQ ID NO: 16 - protein, 16 aa, synthetic construct
HRRCNPNNKKRVPALR

SEQ ID NO: 17 - protein, 19 aa, synthetic construct
VSRRRRRRGGRRRRVPALR

SEQ ID NO: 18 - protein, 20 aa, synthetic construct
GKCSTRGRKCCRRKKVPALR

SEQ ID NO: 19 - protein, 27 aa, synthetic construct
LRRERQSRLRRERQSRHRRCNKNNKKR

SEQ ID NO: 20 - protein, 27 aa, synthetic construct
LRRERQSRLRRERQSRHRRCNPNNKKR

SEQ ID NO: 21 - protein, 30 aa, synthetic construct
LRRERQSRLRRERQSRVSRRRRRRGGRRRR

SEQ ID NO: 22 - protein, 31 aa, synthetic construct
LRRERQSRLRRERQSRGKCSTRGRKCCRRKK

SEQ ID NO: 23 - protein, 27 aa, synthetic construct
HRRCNKNNKKRLRRERQSRLRRERQSR

SEQ ID NO: 24 - protein, 27 aa, synthetic construct
HRRCNPNNKKRLRRERQSRLRRERQSR

SEQ ID NO: 25 - protein, 30 aa, synthetic construct
VSRRRRRRGGRRRRLRRERQSRLRRERQSR

SEQ ID NO: 26 - protein, 31 aa, synthetic construct
GKCSTRGRKCCRRKKLRRERQSRLRRERQSR

SEQ ID NO: 27 - protein, 30 aa, synthetic construct
VPALRRERQSRLRRERQSRHRRCNKNNKKR

SEQ ID NO: 28 - protein, 30 aa, synthetic construct
VPALRRERQSRLRRERQSRHRRCNPNNKKR

SEQ ID NO: 29 - protein, 33 aa, synthetic construct
VPALRRERQSRLRRERQSRVSRRRRRRGGRRRR

SEQ ID NO: 30 - protein, 34 aa, synthetic construct
VPALRRERQSRLRRERQSRGKCSTRGRKCCRRKK

SEQ ID NO: 31 - protein, 30 aa, synthetic construct
HRRCNKNNKKRVPALRRERQSRLRRERQSR

SEQ ID NO: 32 - protein, 30 aa, synthetic construct
HRRCNPNNKKRVPALRRERQSRLRRERQSR

SEQ ID NO: 33 - protein, 33 aa, synthetic construct
VSRRRRRRGGRRRRVPALRRERQSRLRRERQSR

SEQ ID NO: 34 - protein, 34 aa, synthetic construct
GKCSTRGRKCCRRKKVPALRRERQSRLRRERQSR

SEQ ID NO: 35 - protein, 18 aa, synthetic construct
HAIYPRHHRRCNKNNKKR

SEQ ID NO: 36 - protein, 18 aa, synthetic construct
HAIYPRHHRRCNPNNKKR

SEQ ID NO: 37 - protein, 21 aa, synthetic construct
HAIYPRHVSRRRRRRGGRRRR

SEQ ID NO: 38 - protein, 22 aa, synthetic construct
HAIYPRHGKCSTRGRKCCRRKK

SEQ ID NO: 39 - protein, 18 aa, synthetic construct
HRRCNKNNKKRHAIYPRH

SEQ ID NO: 40 - protein, 18 aa, synthetic construct
HRRCNPNNKKRHAIYPRH

SEQ ID NO: 41 - protein, 21 aa, synthetic construct
VSRRRRRRGGRRRRHAIYPRH

SEQ ID NO: 42 - protein, 22 aa, synthetic construct
GKCSTRGRKCCRRKKHAIYPRH

SEQ ID NO: 43 - protein, 23 aa, synthetic construct
YHFNGCEDPLCRHRRCNKNNKKR

SEQ ID NO: 44 - protein, 23 aa, synthetic construct
YHFNGCEDPLCRHRRCNPNNKKR

SEQ ID NO: 45 - protein, 26 aa, synthetic construct
YHFNGCEDPLCRVSRRRRRRGGRRRR

SEQ ID NO: 46 - protein, 27 aa, synthetic construct
YHFNGCEDPLCRGKCSTRGRKCCRRKK

SEQ ID NO: 47 - protein, 23 aa, synthetic construct
HRRCNKNNKKRYHFNGCEDPLCR

SEQ ID NO: 48 - protein, 23 aa, synthetic construct
HRRCNPNNKKRYHFNGCEDPLCR

SEQ ID NO: 49 - protein, 26 aa, synthetic construct
VSRRRRRRGGRRRRYHFNGCEDPLCR

SEQ ID NO: 50 - protein, 27 aa, synthetic construct
GKCSTRGRKCCRRKKYHFNGCEDPLCR

SEQ ID NO: 51 - protein, 23 aa, synthetic construct
HPWCCGLRLDLRHRRCNKNNKKR

SEQ ID NO: 52 - protein, 23 aa, synthetic construct
HPWCCGLRLDLRHRRCNPNNKKR

SEQ ID NO: 53 - protein, 26 aa, synthetic construct
HPWCCGLRLDLRVSRRRRRRGGRRRR

SEQ ID NO: 54 - protein, 27 aa, synthetic construct
HPWCCGLRLDLRGKCSTRGRKCCRRKK

SEQ ID NO: 55 - protein, 23 aa, synthetic construct
HRRCNKNNKKRHPWCCGLRLDLR

SEQ ID NO: 56 - protein, 23 aa, synthetic construct
HRRCNPNNKKRHPWCCGLRLDLR

SEQ ID NO: 57 - protein, 26 aa, synthetic construct
VSRRRRRRGGRRRRHPWCCGLRLDLR

SEQ ID NO: 58 - protein, 27 aa, synthetic construct
GKCSTRGRKCCRRKKHPWCCGLRLDLR

SEQ ID NO: 59 - protein, 272 aa, synthetic construct
MAWVWTLLFLMAAAQSIQAEWIKQRPGQGLEWIGVIHPGNGGTNYNENFKGKATLTADKSSSTAYMQLSSLTSDDSAVYFCASGNDGSYWGQGTTVTVSSGGGGSGKGGSGGGGSGGGGSDIELTQSPSSLTVTAGEKVTMSCKSSQSLLNSGDQKIYLTWYQQKPGQPPKLLIYWASTRESGVPDRFTGSVSGTDFTLTISSVQAEDLAVYYCQNDYNYPYTFGGGTKCLEIKRGSENLYFQGGSGKPIPNPLLGLDSTGGSGGSHHHHHH

SEQ ID NO: 60 - RNA, 20 nt, synthetic construct
  source 1..20: mol_type = other RNA
gtgcaatgaagggaccagta

SEQ ID NO: 61 - RNA, 19 nt, synthetic construct
  source 1..19: mol_type = other RNA
tactggtccctcattgcac

SEQ ID NO: 62 - protein, 33 aa, synthetic construct
CPISQVHEIGIKRNMTVHFKVLREEGPAHMKNF

SEQ ID NO: 63 - protein, 13 aa, synthetic construct
CPISQVHEIGIKR

SEQ ID NO: 64 - protein, 14 aa, synthetic construct
CNMTVHFKVLREEG

SEQ ID NO: 65 - protein, 11 aa, synthetic construct
CPAHMKNFITA

SEQ ID NO: 66 - protein, 26 aa, synthetic construct
CIVTEGEGNGKKVSKKRAAEKMLVEL

SEQ ID NO: 67 - protein, 14 aa, synthetic construct
CEGNGKKVSKKRAA

SEQ ID NO: 68 - protein, 30 aa, synthetic construct
EEEGEEEGEGGGGGHRRCNKNNKKRVPALR

SEQ ID NO: 69 - protein, 35 aa, synthetic construct
EEEGEEEGEGGGGGHRRCNPNNKKRGGGGGVPALR

SEQ ID NO: 70 - protein, 38 aa, synthetic construct
EEEGEEEGEGGGGGVSRRRRRRGGRRRRGGGGGVPALR

SEQ ID NO: 71 - protein, 39 aa, synthetic construct
EEEGEEEGEGGGGGGKCSTRGRKCCRRKKGGGGGVPALR

SEQ ID NO: 72 - protein, 41 aa, synthetic construct
EEEGEEEGEGGGGGHRRCNKNNKKRLRRERQSRLRRERQSR

SEQ ID NO: 73 - protein, 41 aa, synthetic construct
EEEGEEEGEGGGGGHRRCNPNNKKRLRRERQSRLRRERQSR

SEQ ID NO: 74 - protein, 49 aa, synthetic construct
EEEGEEEGEGGGGGVSRRRRRRGGRRRRGGGGGLRRERQSRLRRERQSR

SEQ ID NO: 75 - protein, 45 aa, synthetic construct
EEEGEEEGEGGGGGGKCSTRGRKCCRRKKLRRERQSRLRRERQSR

SEQ ID NO: 76 - protein, 44 aa, synthetic construct
EEEGEEEGEGGGGGHRRCNKNNKKRVPALRRERQSRLRRERQSR

SEQ ID NO: 77 - protein, 44 aa, synthetic construct
EEEGEEEGEGGGGGHRRCNPNNKKRVPALRRERQSRLRRERQSR

SEQ ID NO: 78 - protein, 47 aa, synthetic construct
EEEGEEEGEGGGGGVSRRRRRRGGRRRRVPALRRERQSRLRRERQSR

SEQ ID NO: 79 - protein, 48 aa, synthetic construct
EEEGEEEGEGGGGGGKCSTRGRKCCRRKKVPALRRERQSRLRRERQSR

SEQ ID NO: 80 - protein, 32 aa, synthetic construct
EEEGEEEGEGGGGGHRRCNKNNKKRHAIYPRH

SEQ ID NO: 81 - protein, 32 aa, synthetic construct
EEEGEEEGEGGGGGHRRCNPNNKKRHAIYPRH

SEQ ID NO: 82 - protein, 35 aa, synthetic construct
EEEGEEEGEGGGGGVSRRRRRRGGRRRRHAIYPRH

SEQ ID NO: 83 - protein, 36 aa, synthetic construct
EEEGEEEGEGGGGGGKCSTRGRKCCRRKKHAIYPRH

SEQ ID NO: 84 - protein, 45 aa, synthetic construct
EEEGEEEGEGGGGGVSRRRRRRGGRRRRGGGGGYHFNGCEDPLCR

SEQ ID NO: 85 - protein, 45 aa, synthetic construct
EEEGEEEGEGGGGGVSRRRRRRGGRRRRGGGGGHPWCCGLRLDLR

SEQ ID NO: 86 - DNA, 22 bp, Mus musculus
  source 1..22: mol_type = other DNA
gtatgactccactcacggcaaa

SEQ ID NO: 87 - DNA, 20 bp, Mus musculus
  source 1..20: mol_type = other DNA
ggtctcgctcctggaagatg

SEQ ID NO: 88 - DNA, 22 bp, Mus musculus
  source 1..22: mol_type = other DNA
gatattgacgggcagtatgcaa

SEQ ID NO: 89 - DNA, 20 bp, Mus musculus
  source 1..20: mol_type = other DNA
aactgcgtggatgggatctg